European Patent Application EP 4 242 220 A1, published September 13, 2023. Title: Peptide crosslinking agent and paptide crosslinked by the agent. Applicant: Kagoshima University. The sequence listing filed with the application follows.

SEQUENCE LISTING (78 sequences)

SEQ ID NO: 1 - protein, 22 aa, Artificial Sequence
  Fc binding peptide
GSGGSGPDCAYHRGELVWCTFH

SEQ ID NO: 2 - protein, 35 aa, Artificial Sequence
  Fc binding peptide
  MISC_FEATURE (1)..(1): X is G, A, V, L, I, M, P, F, W, K, Orn, C, D, E, Dpr, or 2-Aminooctanedioic acid
  MISC_FEATURE (2)..(2): X is F,K,Orn,C,D,E,2-Aminooctanedioic acid, or Dpr
  misc_feature (27)..(27): Xaa can be any naturally occurring amino acid
  MISC_FEATURE (29)..(29): X is R,H,D,E,S,T,N,Q,Y, or C
  MISC_FEATURE (31)..(31): X is R,H,D,E,S,T,N,Q,Y, or C
XXNMQCQRRFYEALHDPNLNEEQRNAXIXSIRDDC

SEQ ID NO: 3 - protein, 35 aa, Artificial Sequence
  Ig binding peptide
  MISC_FEATURE (1)..(1): X is G, A, V, L, I, M, P, F, W, K, Orn, C, D, E, Dpr, or 2-Aminooctanedioic acid
  MISC_FEATURE (2)..(2): X is F,K,Orn,C,D,E,2-Aminooctanedioic acid, or Dpr
  MISC_FEATURE (8)..(8): X is R, C, or K
  misc_feature (27)..(27): Xaa can be any naturally occurring amino acid
  MISC_FEATURE (29)..(29): X is X is R,H,D,E,S,T,N,Q,Y, or C
  MISC_FEATURE (31)..(31): X is R,H,D,E,S,T,N,Q,Y, or C
XXNMQCQXRFYEALHDPNLNEEQRNAXIXSIRDDC

SEQ ID NO: 4 - protein, 13 aa, Artificial Sequence
  IgG-BP
  MISC_FEATURE (6)..(6): X is K, C, D, E, R, V, F, L, 2-Aminosuberic acid, Dpr, Orn, AcOrn, AcDab, Dab, Nle, Nva, Tle, Ala(t-Bu), or Cha
DCAYHXGELVWCT

SEQ ID NO: 5 - protein, 17 aa, Artificial Sequence
  IgG-BP
  MISC_FEATURE (8)..(8): X is K, C, D, E, R, V, F, L, 2-Aminosuberic acid, Dpr, Orn, AcOrn, AcDab, Dab, Nle, Nva, Tle, Ala(t-Bu), or Cha
GPDCAYHXGELVWCTFH

SEQ ID NO: 6 - protein, 13 aa, Artificial Sequence
  IgG-BP
  MISC_FEATURE (6)..(6): X is K, C, D, E, R, V, F, L, 2-Aminosuberic acid, Dpr, Orn, AcOrn, AcDab, Dab, Nle, Nva, Tle, Ala(t-Bu), or Cha
RCAYHXGELVWCS

SEQ ID NO: 7 - protein, 17 aa, Artificial Sequence
  IgG-BP
  MISC_FEATURE (8)..(8): X is K, C, D, E, R, V, F, L, 2-Aminosuberic acid, Dpr, Orn, AcOrn, AcDab, Dab, Nle, Nva, Tle, Ala(t-Bu), or Cha
GPRCAYHXGELVWCSFH

SEQ ID NO: 8 - protein, 17 aa, Artificial Sequence
  IgG-BP
  MISC_FEATURE (8)..(8): X is K, C, D, E, R, V, F, L, 2-Aminosuberic acid, Dpr, Orn, AcOrn, AcDab, Dab, Nle, Nva, Tle, Ala(t-Bu), or Cha
SPDCAYHXGELVWCTFH

SEQ ID NO: 9 - protein, 17 aa, Artificial Sequence
  IgG-BP
  MISC_FEATURE (8)..(8): X is K,C,D,E, R, 2-Aminosuberic acid, or Diaminopropionic acid
GDDCAYHXGELVWCTFH

SEQ ID NO: 10 - protein, 17 aa, Artificial Sequence
  IgG-BP
  MISC_FEATURE (8)..(8): X is K, C, D, E, R, V, F, L, 2-Aminosuberic acid, Dpr, Orn, AcOrn, AcDab, Dab, Nle, Nva, Tle, Ala(t-Bu), or Cha
GPSCAYHXGELVWCTFH

SEQ ID NO: 11 - protein, 17 aa, Artificial Sequence
  IgG-BP
  MISC_FEATURE (8)..(8): X is K, C, D, E, R, V, F, L, 2-Aminosuberic acid, Dpr, Orn, AcOrn, AcDab, Dab, Nle, Nva, Tle, Ala(t-Bu), or Cha
GPDCAYHXGELVWCSFH

SEQ ID NO: 12 - protein, 17 aa, Artificial Sequence
  IgG-BP
  MISC_FEATURE (8)..(8): X is K, C, D, E, R, V, F, L, 2-Aminosuberic acid, Dpr, Orn, AcOrn, AcDab, Dab, Nle, Nva, Tle, Ala(t-Bu), or Cha
GPDCAYHXGELVWCTHH

SEQ ID NO: 13 - protein, 17 aa, Artificial Sequence
  IgG-BP
  MISC_FEATURE (8)..(8): X is K, C, D, E, R, V, F, L, 2-Aminosuberic acid, Dpr, Orn, AcOrn, AcDab, Dab, Nle, Nva, Tle, Ala(t-Bu), or Cha
GPDCAYHXGELVWCTFY

SEQ ID NO: 14 - protein, 17 aa, Artificial Sequence
  IgG-BP
  MISC_FEATURE (8)..(8): X is K, C, D, E, R, V, F, L, 2-Aminosuberic acid, Dpr, Orn, AcOrn, AcDab, Dab, Nle, Nva, Tle, Ala(t-Bu), or Cha
SPDCAYHXGELVWCTFY

SEQ ID NO: 15 - protein, 17 aa, Artificial Sequence
  IgG-BP
  MISC_FEATURE (8)..(8): X is K, C, D, E, R, V, F, L, 2-Aminosuberic acid, Dpr, Orn, AcOrn, AcDab, Dab, Nle, Nva, Tle, Ala(t-Bu), or Cha
SDDCAYHXGELVWCTFY

SEQ ID NO: 16 - protein, 17 aa, Artificial Sequence
  IgG-BP
  MISC_FEATURE (8)..(8): X is K, C, D, E, R, V, F, L, 2-Aminosuberic acid, Dpr, Orn, AcOrn, AcDab, Dab, Nle, Nva, Tle, Ala(t-Bu), or Cha
RGNCAYHXGQLVWCTYH

SEQ ID NO: 17 - protein, 17 aa, Artificial Sequence
  IgG-BP
  MISC_FEATURE (2)..(2): X is homocysteine
  MISC_FEATURE (8)..(8): X is K, C, D, E, R, V, F, L, 2-Aminosuberic acid, Dpr, Orn, AcOrn, AcDab, Dab, Nle, Nva, Tle, Ala(t-Bu), or Cha
  misc_feature (16)..(16): Xaa can be any naturally occurring amino acid
  MISC_FEATURE (17)..(17): X is homocysteine
GXDCAYHXGELVWCTXH

SEQ ID NO: 18 - protein, 19 aa, Artificial Sequence
  IgG-BP
  MISC_FEATURE (10)..(10): X is K, C, D, E, R, V, F, L, 2-Aminosuberic acid, Dpr, Orn, AcOrn, AcDab, Dab, Nle, Nva, Tle, Ala(t-Bu), or Cha
RRGPDCAYHXGELVWCTFH

SEQ ID NO: 19 - protein, 13 aa, Artificial Sequence
  IgG-BP
  MISC_FEATURE (6)..(6): X is K, C, D, E, R, V, F, L, 2-Aminosuberic acid, Dpr, Orn, AcOrn, AcDab, Dab, Nle, Nva, Tle, Ala(t-Bu), or Cha
DCTYHXGNLVWCT

SEQ ID NO: 20 - protein, 13 aa, Artificial Sequence
  IgG-BP
  MISC_FEATURE (6)..(6): X is K, C, D, E, R, V, F, L, 2-Aminosuberic acid, Dpr, Orn, AcOrn, AcDab, Dab, Nle, Nva, Tle, Ala(t-Bu), or Cha
DCAYHXGNLVWCT

SEQ ID NO: 21 - protein, 13 aa, Artificial Sequence
  IgG-BP
  MISC_FEATURE (6)..(6): X is K, C, D, E, R, V, F, L, 2-Aminosuberic acid, Dpr, Orn, AcOrn, AcDab, Dab, Nle, Nva, Tle, Ala(t-Bu), or Cha
DCTYHXGELVWCT

SEQ ID NO: 22 - protein, 13 aa, Artificial Sequence
  IgG-BP
  MISC_FEATURE (6)..(6): X is K, C, D, E, R, V, F, L, 2-Aminosuberic acid, Dpr, Orn, AcOrn, AcDab, Dab, Nle, Nva, Tle, Ala(t-Bu), or Cha
DCAWHXGELVWCT

SEQ ID NO: 23 - protein, 13 aa, Artificial Sequence
  IgG-BP
  MISC_FEATURE (6)..(6): X is K, C, D, E, R, V, F, L, 2-Aminosuberic acid, Dpr, Orn, AcOrn, AcDab, Dab, Nle, Nva, Tle, Ala(t-Bu), or Cha
DCTYTXGNLVWCT

SEQ ID NO: 24 - protein, 13 aa, Artificial Sequence
  IgG-BP
  MISC_FEATURE (6)..(6): X is K, C, D, E, R, V, F, L, 2-Aminosuberic acid, Dpr, Orn, AcOrn, AcDab, Dab, Nle, Nva, Tle, Ala(t-Bu), or Cha
DCAYTXGNLVWCT

SEQ ID NO: 25 - protein, 13 aa, Artificial Sequence
  IgG-BP
  MISC_FEATURE (6)..(6): X is K, C, D, E, R, V, F, L, 2-Aminosuberic acid, Dpr, Orn, AcOrn, AcDab, Dab, Nle, Nva, Tle, Ala(t-Bu), or Cha
DCSYTXGNLVWCT

SEQ ID NO: 26 - protein, 13 aa, Artificial Sequence
  IgG-BP
  MISC_FEATURE (6)..(6): X is K, C, D, E, R, V, F, L, 2-Aminosuberic acid, Dpr, Orn, AcOrn, AcDab, Dab, Nle, Nva, Tle, Ala(t-Bu), or Cha
DCTWTXGNLVWCT

SEQ ID NO: 27 - protein, 13 aa, Artificial Sequence
  IgG-BP
  MISC_FEATURE (6)..(6): X is K, C, D, E, R, V, F, L, 2-Aminosuberic acid, Dpr, Orn, AcOrn, AcDab, Dab, Nle, Nva, Tle, Ala(t-Bu), or Cha
DCTYHXGNLVWCT

SEQ ID NO: 28 - protein, 13 aa, Artificial Sequence
  IgG-BP
  MISC_FEATURE (6)..(6): X is K, C, D, E, R, V, F, L, 2-Aminosuberic acid, Dpr, Orn, AcOrn, AcDab, Dab, Nle, Nva, Tle, Ala(t-Bu), or Cha
DCTYRXGNLVWCT

SEQ ID NO: 29 - protein, 13 aa, Artificial Sequence
  IgG-BP
  MISC_FEATURE (6)..(6): X is K, C, D, E, R, V, F, L, 2-Aminosuberic acid, Dpr, Orn, AcOrn, AcDab, Dab, Nle, Nva, Tle, Ala(t-Bu), or Cha
DCTYSXGNLVWCT

SEQ ID NO: 30 - protein, 13 aa, Artificial Sequence
  IgG-BP
  MISC_FEATURE (6)..(6): X is K, C, D, E, R, V, F, L, 2-Aminosuberic acid, Dpr, Orn, AcOrn, AcDab, Dab, Nle, Nva, Tle, Ala(t-Bu), or Cha
DCTYTXGNLVWCT

SEQ ID NO: 31 - protein, 13 aa, Artificial Sequence
  IgG-BP
  MISC_FEATURE (6)..(6): X is K, C, D, E, R, V, F, L, 2-Aminosuberic acid, Dpr, Orn, AcOrn, AcDab, Dab, Nle, Nva, Tle, Ala(t-Bu), or Cha
DCTYTXGELVWCT

SEQ ID NO: 32 - protein, 13 aa, Artificial Sequence
  IgG-BP
  MISC_FEATURE (6)..(6): X is K, C, D, E, R, V, F, L, 2-Aminosuberic acid, Dpr, Orn, AcOrn, AcDab, Dab, Nle, Nva, Tle, Ala(t-Bu), or Cha
DCTYTXGRLVWCT

SEQ ID NO: 33 - protein, 13 aa, Artificial Sequence
  IgG-BP
  MISC_FEATURE (6)..(6): X is K, C, D, E, R, V, F, L, 2-Aminosuberic acid, Dpr, Orn, AcOrn, AcDab, Dab, Nle, Nva, Tle, Ala(t-Bu), or Cha
DCTYTXGDLVWCT

SEQ ID NO: 34 - protein, 13 aa, Artificial Sequence
  IgG-BP
  MISC_FEATURE (6)..(6): X is K, C, D, E, R, V, F, L, 2-Aminosuberic acid, Dpr, Orn, AcOrn, AcDab, Dab, Nle, Nva, Tle, Ala(t-Bu), or Cha
DCTYTXGNLIWCT

SEQ ID NO: 35 - protein, 13 aa, Artificial Sequence
  IgG-BP
DCAYHRGELVWCT

SEQ ID NO: 36 - protein, 17 aa, Artificial Sequence
  IgG-BP
GPDCAYHRGELVWCTFH

SEQ ID NO: 37 - protein, 13 aa, Artificial Sequence
  IgG-BP
RCAYHRGELVWCS

SEQ ID NO: 38 - protein, 17 aa, Artificial Sequence
  IgG-BP
GPRCAYHRGELVWCSFH

SEQ ID NO: 39 - protein, 17 aa, Artificial Sequence
  IgG-BP
SPDCAYHRGELVWCTFH

SEQ ID NO: 40 - protein, 17 aa, Artificial Sequence
  IgG-BP
GDDCAYHRGELVWCTFH

SEQ ID NO: 41 - protein, 17 aa, Artificial Sequence
  IgG-BP
GPSCAYHRGELVWCTFH

SEQ ID NO: 42 - protein, 17 aa, Artificial Sequence
  IgG-BP
GPDCAYHRGELVWCSFH

SEQ ID NO: 43 - protein, 17 aa, Artificial Sequence
  IgG-BP
GPDCAYHRGELVWCTHH

SEQ ID NO: 44 - protein, 17 aa, Artificial Sequence
  IgG-BP
GPDCAYHRGELVWCTFY

SEQ ID NO: 45 - protein, 17 aa, Artificial Sequence
  IgG-BP
SPDCAYHRGELVWCTFY

SEQ ID NO: 46 - protein, 17 aa, Artificial Sequence
  IgG-BP
SDDCAYHRGELVWCTFY

SEQ ID NO: 47 - protein, 13 aa, Artificial Sequence
  IgG-BP
DCTYHRGNLVWCT

SEQ ID NO: 48 - protein, 13 aa, Artificial Sequence
  IgG-BP
DCAYHRGNLVWCT

SEQ ID NO: 49 - protein, 13 aa, Artificial Sequence
  IgG-BP
DCTYHRGELVWCT

SEQ ID NO: 50 - protein, 13 aa, Artificial Sequence
  IgG-BP
DCAWHRGELVWCT

SEQ ID NO: 51 - protein, 13 aa, Artificial Sequence
  IgG-BP
DCTYTNGNLVWCT

SEQ ID NO: 52 - protein, 13 aa, Artificial Sequence
  IgG-BP
DCAYTNGNLVWCT

SEQ ID NO: 53 - protein, 13 aa, Artificial Sequence
  IgG-BP
DCSYTNGNLVWCT

SEQ ID NO: 54 - protein, 13 aa, Artificial Sequence
  IgG-BP
DCTWTNGNLVWCT

SEQ ID NO: 55 - protein, 13 aa, Artificial Sequence
  IgG-BP
DCTYHNGNLVWCT

SEQ ID NO: 56 - protein, 13 aa, Artificial Sequence
  IgG-BP
DCTYRNGNLVWCT

SEQ ID NO: 57 - protein, 13 aa, Artificial Sequence
  IgG-BP
DCTYSNGNLVWCT

SEQ ID NO: 58 - protein, 13 aa, Artificial Sequence
  IgG-BP
DCTYTRGNLVWCT

SEQ ID NO: 59 - protein, 13 aa, Artificial Sequence
  IgG-BP
DCTYTNGELVWCT

SEQ ID NO: 60 - protein, 13 aa, Artificial Sequence
  IgG-BP
DCTYTNGRLVWCT

SEQ ID NO: 61 - protein, 13 aa, Artificial Sequence
  IgG-BP
DCTYTNGDLVWCT

SEQ ID NO: 62 - protein, 13 aa, Artificial Sequence
  IgG-BP
DCTYTNGNLIWCT

SEQ ID NO: 63 - protein, 34 aa, Artificial Sequence
  IgG-BP
FNMQCQRRFYEALHDPNLNEEQRNARIRSIRDDC

SEQ ID NO: 64 - protein, 35 aa, Artificial Sequence
  IgG-BP
GFNMQCQRRFYEALHDPNLNEEQRNARIRSIRDDC

SEQ ID NO: 65 - protein, 34 aa, Artificial Sequence
  IgG-BP
KNMQCQRRFYEALHDPNLNEEQRNARIRSIRDDC

SEQ ID NO: 66 - protein, 35 aa, Artificial Sequence
  IgG-BP
GFNMQCQKRFYEALHDPNLNEEQRNARIRSIRDDC

SEQ ID NO: 67 - protein, 34 aa, Artificial Sequence
  IgG-BP
KNMQCQKRFYEALHDPNLNEEQRNARIRSIRDDC

SEQ ID NO: 68 - protein, 33 aa, Artificial Sequence
  IgG-BP
FNMQQQRRFYEALHDPNLNEEQRNARIRSIRDD

SEQ ID NO: 69 - protein, 35 aa, Artificial Sequence
  IgG-BP
GKNMQCQRRFYEALHDPNLNEEQRNARIRSIRDDC

SEQ ID NO: 70 - protein, 11 aa, Artificial Sequence
  Fc binding peptide
CAWHLGELVWC

SEQ ID NO: 71 - protein, 13 aa, Artificial Sequence
  Fc binding peptide
DCAWHLGELVWCT

SEQ ID NO: 72 - protein, 13 aa, Artificial Sequence
  Fc binding peptide
DCAWHLGELVFCT

SEQ ID NO: 73 - protein, 10 aa, Artificial Sequence
  Fc binding peptide
DCAWHLGELV

SEQ ID NO: 74 - protein, 15 aa, Artificial Sequence
  Fc binding peptide
CDCAWHLGELVWCTC

SEQ ID NO: 75 - protein, 11 aa, Artificial Sequence
  Fc binding peptide
CAYHLGELVWC

SEQ ID NO: 76 - protein, 14 aa, Artificial Sequence
  Fc binding peptide
DCAYHLGELVWCTF

SEQ ID NO: 77 - protein, 9 aa, Homo sapiens
CYIQNCPLG

SEQ ID NO: 78 - protein, 9 aa, Homo sapiens
CYFQNCPRG